European Patent Application EP 4 368 185 A1, published May 15, 2024. Title: Combination of Menin inhibitor(s) and Immunoprotease inhibitor(s) for treatment of leukemia. Applicant: Universitätsmedizin Greifswald. The sequence listing filed with the application follows.

SEQUENCE LISTING (34 sequences)

SEQ ID NO: 1 - RNA, 20 nt, synthetic construct
  misc_feature 1..20: note = Luciferase sgRNA
  source 1..20: mol_type = other RNA
gattctaaaacggattacca

SEQ ID NO: 2 - RNA, 20 nt, synthetic construct
  misc_feature 1..20: note = RPA3 sgRNA1
  source 1..20: mol_type = other RNA
ggttggaagagtaaccgcca

SEQ ID NO: 3 - RNA, 20 nt, synthetic construct
  misc_feature 1..20: note = RPA3 sgRNA2
  source 1..20: mol_type = other RNA
gatgaattgagctagcatgc

SEQ ID NO: 4 - RNA, 20 nt, synthetic construct
  misc_feature 1..20: note = PSMB5 sgRNA1
  source 1..20: mol_type = other RNA
tttgtactgatacaccatgt

SEQ ID NO: 5 - RNA, 20 nt, synthetic construct
  misc_feature 1..20: note = PSMB5 sgRNA2
  source 1..20: mol_type = other RNA
gcttcatggaacaaccaccc

SEQ ID NO: 6 - RNA, 20 nt, synthetic construct
  misc_feature 1..20: note = PSMB5 sgRNA3
  source 1..20: mol_type = other RNA
ccgctaccggtgaaccagcg

SEQ ID NO: 7 - RNA, 20 nt, synthetic construct
  misc_feature 1..20: note = PSMB5 sgRNA4
  source 1..20: mol_type = other RNA
tgcttacattgcctcccaga

SEQ ID NO: 8 - RNA, 20 nt, synthetic construct
  misc_feature 1..20: note = PSMB8 sgRNA1
  source 1..20: mol_type = other RNA
ccagagctcgctttaccccg

SEQ ID NO: 9 - RNA, 20 nt, synthetic construct
  misc_feature 1..20: note = PSMB8 sgRNA2
  source 1..20: mol_type = other RNA
aaggaacgttcagattgaga

SEQ ID NO: 10 - RNA, 20 nt, synthetic construct
  misc_feature 1..20: note = PSMB8 sgRNA3
  source 1..20: mol_type = other RNA
ccggtactggcacatcatgt

SEQ ID NO: 11 - RNA, 20 nt, synthetic construct
  misc_feature 1..20: note = PSMB8 sgRNA4
  source 1..20: mol_type = other RNA
aggtgccttacgggtgaaca

SEQ ID NO: 12 - RNA, 20 nt, synthetic construct
  misc_feature 1..20: note = PSMB8 sgRNA5
  source 1..20: mol_type = other RNA
tgtggctgggataagaaggt

SEQ ID NO: 13 - RNA, 20 nt, synthetic construct
  misc_feature 1..20: note = PSMB9 sgRNA1
  source 1..20: mol_type = other RNA
gtagatgcgctcgtgcagcg

SEQ ID NO: 14 - RNA, 20 nt, synthetic construct
  misc_feature 1..20: note = PSMB9 sgRNA3
  source 1..20: mol_type = other RNA
tcccagggttccatatacct

SEQ ID NO: 15 - RNA, 20 nt, synthetic construct
  misc_feature 1..20: note = PSMB9 sgRNA4
  source 1..20: mol_type = other RNA
gcagcagccaaaacaagtgg

SEQ ID NO: 16 - RNA, 20 nt, synthetic construct
  misc_feature 1..20: note = PSMB10 sgRNA1
  source 1..20: mol_type = other RNA
cactaacgattcggtcgtgg

SEQ ID NO: 17 - RNA, 20 nt, synthetic construct
  misc_feature 1..20: note = PSMB10 sgRNA2
  source 1..20: mol_type = other RNA
cgatcagcgatgcacccacg

SEQ ID NO: 18 - RNA, 20 nt, synthetic construct
  misc_feature 1..20: note = PSMB10 sgRNA3
  source 1..20: mol_type = other RNA
tgtggtcatctcggcgtccg

SEQ ID NO: 19 - RNA, 21 nt, synthetic construct
  misc_feature 1..21: note = BASP1_Fw
  source 1..21: mol_type = other RNA
aggggaacccaaaaagactga

SEQ ID NO: 20 - RNA, 20 nt, synthetic construct
  misc_feature 1..20: note = BASP1_Rv
  source 1..20: mol_type = other RNA
ggtgtggaactaggcgcttc

SEQ ID NO: 21 - RNA, 18 nt, synthetic construct
  misc_feature 1..18: note = PSMB5_Fw
  source 1..18: mol_type = other RNA
gctaccggtgaaccagcg

SEQ ID NO: 22 - RNA, 21 nt, synthetic construct
  misc_feature 1..21: note = PSMB5_Rv
  source 1..21: mol_type = other RNA
caactatgactccatggcgga

SEQ ID NO: 23 - RNA, 20 nt, synthetic construct
  misc_feature 1..20: note = PSMB6_Fw
  source 1..20: mol_type = other RNA
cactccagactgggaaagcc

SEQ ID NO: 24 - RNA, 20 nt, synthetic construct
  misc_feature 1..20: note = PSMB6_Rv
  source 1..20: mol_type = other RNA
gacagcagaaaatgcggtcg

SEQ ID NO: 25 - RNA, 20 nt, synthetic construct
  misc_feature 1..20: note = PSMB7_Fw
  source 1..20: mol_type = other RNA
cacagacatgacaacccagc

SEQ ID NO: 26 - RNA, 20 nt, synthetic construct
  misc_feature 1..20: note = PSMB7_Rv
  source 1..20: mol_type = other RNA
agggctgcaccaatgtaacc

SEQ ID NO: 27 - RNA, 21 nt, synthetic construct
  misc_feature 1..21: note = PSMB8_Fw
  source 1..21: mol_type = other RNA
ccttacctgcttggcaccatg

SEQ ID NO: 28 - RNA, 21 nt, synthetic construct
  misc_feature 1..21: note = PSMB8_Rv
  source 1..21: mol_type = other RNA
ttggaggctgccgacactgaa

SEQ ID NO: 29 - RNA, 20 nt, synthetic construct
  misc_feature 1..20: note = PSMB9_Fw
  source 1..20: mol_type = other RNA
ggcgttgtgatgggttctga

SEQ ID NO: 30 - RNA, 21 nt, synthetic construct
  misc_feature 1..21: note = PSMB9_Rv
  source 1..21: mol_type = other RNA
agagagtgcacagtagatgcg

SEQ ID NO: 31 - RNA, 21 nt, synthetic construct
  misc_feature 1..21: note = PSMB10_Fw
  source 1..21: mol_type = other RNA
agctacacgcgttatctacgg

SEQ ID NO: 32 - RNA, 20 nt, synthetic construct
  misc_feature 1..20: note = PSMB10_Rv
  source 1..20: mol_type = other RNA
ctgcggtccagtcaggtcta

SEQ ID NO: 33 - RNA, 24 nt, synthetic construct
  misc_feature 1..24: note = Beta-2-microgobulin_Fw
  source 1..24: mol_type = other RNA
tgtgtctgggtttcatccatccga

SEQ ID NO: 34 - RNA, 24 nt, synthetic construct
  misc_feature 1..24: note = Beta-2-microgobulin_Rv
  source 1..24: mol_type = other RNA
cacacggcaggcatactcatcttt